European Patent Application EP 4 480 494 A1, published December 25, 2024. Title: Composition for Use in Treatment of Cancer, Inflammatory Disease, or Obesity and Use Thereof. Applicant: National University Corporation Tokyo Medical and Dental University. The sequence listing filed with the application follows.

SEQUENCE LISTING (22 sequences)

SEQ ID NO: 1 - DNA, 20 bp, synthetic construct
  source 1..20: mol_type = other DNA
ccaaccttctggttgagctg

SEQ ID NO: 2 - DNA, 22 bp, synthetic construct
  source 1..22: mol_type = other DNA
catccagggaaaacaacacaga

SEQ ID NO: 3 - DNA, 20 bp, synthetic construct
  source 1..20: mol_type = other DNA
gatgacctgccaacagacca

SEQ ID NO: 4 - DNA, 20 bp, synthetic construct
  source 1..20: mol_type = other DNA
gtcctcttcaggtgcctcag

SEQ ID NO: 5 - DNA, 20 bp, synthetic construct
  source 1..20: mol_type = other DNA
aactggaacccagaagcaca

SEQ ID NO: 6 - DNA, 20 bp, synthetic construct
  source 1..20: mol_type = other DNA
cagctgtccctgttgtcgaa

SEQ ID NO: 7 - DNA, 20 bp, synthetic construct
  source 1..20: mol_type = other DNA
cgggacccattcaggatcac

SEQ ID NO: 8 - DNA, 20 bp, synthetic construct
  source 1..20: mol_type = other DNA
cgggacccattcaggatcac

SEQ ID NO: 9 - DNA, 20 bp, synthetic construct
  source 1..20: mol_type = other DNA
ttccctctgaggtgctgtct

SEQ ID NO: 10 - DNA, 24 bp, synthetic construct
  source 1..24: mol_type = other DNA
acatcttgtcatgatcgtccttca

SEQ ID NO: 11 - RNA, 21 nt, synthetic construct
  source 1..21: mol_type = other RNA
agatcgaagagcgtcgtgtag

SEQ ID NO: 12 - DNA, 17 bp, synthetic construct
  source 1..17: mol_type = other DNA
acacgacgctcttccga

SEQ ID NO: 13 - DNA, 32 bp, synthetic construct
  misc_feature 1..10: note = n is a, c, g, or t
  source 1..32: mol_type = other DNA
  misc_feature 1: note = 5 phosphorylation
  misc_feature 32: note = 3 SpC3
nnnnnnnnnnagatcggaagagcacacgtctg

SEQ ID NO: 14 - RNA, 20 nt, synthetic construct
  source 1..20: mol_type = other RNA
actgccgtcgcgtgcagtga

SEQ ID NO: 15 - DNA, 200 bp, synthetic construct
  source 1..200: mol_type = other DNA
agagcaaggagcacccgcagcacctctgcgagaagtgcaaggtcctgggctactactgccgtcgcgtgcaggactacaaggacgacgacgacaaggtgagcggctggcggctgttcaagaagattagctgacgggctgcccgcccgcacccagagccaccccccgccagcccgaggagacgctgcttccctgtgctactc

SEQ ID NO: 16 - RNA, 20 nt, synthetic construct
  source 1..20: mol_type = other RNA
ggtagacccagttgagtagc

SEQ ID NO: 17 - RNA, 22 nt, synthetic construct
  source 1..22: mol_type = other RNA
aatatacatcctccgggatcca

SEQ ID NO: 18 - RNA, 22 nt, synthetic construct
  source 1..22: mol_type = other RNA
aatgtacatcctccgggatcca

SEQ ID NO: 19 - DNA, 23 bp, synthetic construct
  source 1..23: mol_type = other DNA
atgatggcttattacagtggcaa

SEQ ID NO: 20 - DNA, 20 bp, synthetic construct
  source 1..20: mol_type = other DNA
gtcggagattcgtagctgga

SEQ ID NO: 21 - DNA, 21 bp, synthetic construct
  source 1..21: mol_type = other DNA
actgagaggctccgagaaatg

SEQ ID NO: 22 - DNA, 19 bp, synthetic construct
  source 1..19: mol_type = other DNA
gaaccccgcatcttggctt